European Patent Application EP 4 681 721 A1, published January 21, 2026. Title: Recombinant Herpes Simplex Virus with IL-12 Expression. Applicant: TODO, Tomoki. Application JP. The sequence listing filed with the application follows.

SEQUENCE LISTING (13 sequences)

SEQ ID NO: 1 - DNA, 1623 bp, synthetic construct
  source 1..1623: mol_type = other DNA
atgggtcaatcacgctacctcctctttttggccacccttgccctcctaaaccacctcagtttggccagggtcattccagtctctggacctgccaggtgtcttagccagtcccgaaacctgctgaagaccacagatgacatggtgaagacggccagagaaaagctgaaacattattcctgcactgctgaagacatcgatcatgaagacatcacacgggaccaaaccagcacattgaagacctgtttaccactggaactacacaagaacgagagttgcctggctactagagagacttcttccacaacaagagggagctgcctgcccccacagaagacgtctttgatgatgaccctgtgccttggtagcatctatgaggacttgaagatgtaccagacagagttccaggccatcaacgcagcacttcagaatcacaaccatcagcagatcattctagacaagggcatgctggtggccatcgatgagctgatgcagtctctgaatcataatggcgagactctgcgccagaaacctcctgtgggagaagcagacccttacagagtgaaaatgaagctctgcatcctgcttcacgccttcagcacccgcgtcgtgaccatcaacagggtgatgggctatctgagctccgccgttcctggagtaggggtacctggagtgggcggatctatgtgggagctggagaaagacgtttatgttgtagaggtggactggactcccgatgcccctggagaaacagtgaacctcacctgtgacacgcctgaagaagatgacatcacctggacctcagaccagaggcatggagtcataggctctggaaagaccctgaccatcactgtcaaagagtttctagatgctggccagtacacctgccacaaaggaggcgagactctgagccactcacatctgctgctccacaagaaggaaaatggaatttggtccactgaaattttaaaaaatttcaaaaacaagactttcctgaagtgtgaagcaccaaattactccggacggttcacgtgctcatggctggtgcaaagaaacatggacttgaagttcaacatcaagagcagtagcagtccccccgactctcgggcagtgacatgtggaatggcgtctctgtctgcagagaaggtcacactggaccaaagggactatgagaagtattcagtgtcctgccaggaggatgtcacctgcccaactgccgaggagaccctgcccattgaactggcgttggaagcacggcagcagaataaatatgagaactacagcaccagcttcttcatcagggacatcatcaaaccagacccgcccaagaacttgcagatgaagcctttgaagaactcacaggtggaggtcagctgggagtaccctgactcctggagcactccccattcctacttctccctcaagttctttgttcgaatccagcgcaagaaagaaaagatgaaggagacagaggaggggtgtaaccagaaaggtgcgttcctcgtagagaagacatctaccgaagtccaatgcaaaggcgggaatgtctgcgtgcaagctcaggatcgctattacaattcctcatgcagcaagtgggcatgtgttccctgcagggtccgatcctag

SEQ ID NO: 2 - protein, 540 aa, synthetic construct
MGQSRYLLFLATLALLNHLSLARVIPVSGPARCLSQSRNLLKTTDDMVKTAREKLKHYSCTAEDIDHEDITRDQTSTLKTCLPLELHKNESCLATRETSSTTRGSCLPPQKTSLMMTLCLGSIYEDLKMYQTEFQAINAALQNHNHQQIILDKGMLVAIDELMQSLNHNGETLRQKPPVGEADPYRVKMKLCILLHAFSTRVVTINRVMGYLSSAVPGVGVPGVGGSMWELEKDVYVVEVDWTPDAPGETVNLTCDTPEEDDITWTSDQRHGVIGSGKTLTITVKEFLDAGQYTCHKGGETLSHSHLLLHKKENGIWSTEILKNFKNKTFLKCEAPNYSGRFTCSWLVQRNMDLKFNIKSSSSPPDSRAVTCGMASLSAEKVTLDQRDYEKYSVSCQEDVTCPTAEETLPIELALEARQQNKYENYSTSFFIRDIIKPDPPKNLQMKPLKNSQVEVSWEYPDSWSTPHSYFSLKFFVRIQRKKEKMKETEEGCNQKGAFLVEKTSTEVQCKGGNVCVQAQDRYYNSSCSKWACVPCRVRS

SEQ ID NO: 3 - DNA, 1611 bp, synthetic construct
  source 1..1611: mol_type = other DNA
atgggtcaccagcagttggtcatctcttggttttccctggtttttctggcatctcccctcgtggccatatgggaactgaagaaagatgtttatgtcgtagaattggattggtatccggatgcccctggagaaatggtggtcctcacctgtgacacccctgaagaagatggtatcacctggaccttggaccagagcagtgaggtcttaggctctggcaaaaccctgaccatccaagtcaaagagtttggagatgctggccagtacacctgtcacaaaggaggcgaggttctaagccattcgctcctgctgcttcacaaaaaggaagatggaatttggtccactgatattttaaaggaccagaaagaacccaaaaataagacctttctaagatgcgaggccaagaattattctggacgtttcacctgctggtggctgacgacaatcagtactgatttgacattcagtgtcaaaagcagcagaggctcttctgacccccaaggggtgacgtgcggagctgctacactctctgcagagagagtcagaggggacaacaaggagtatgagtactcagtggagtgccaggaggacagtgcctgcccagctgctgaggagagtctgcccattgaggtcatggtggatgccgttcacaagctcaagtatgaaaactacaccagcagcttcttcatcagggacatcatcaaacctgacccacccaagaacttgcagctgaagccattaaagaattctcggcaggtggaggtcagctgggagtaccctgacacctggagtactccacattcctacttctccctgacattctgcgttcaggtccagggcaagagcaagagagaaaagaaagatagagtcttcacggacaagacctcagccacggtcatctgccgcaaaaatgccagcattagcgtgcgggcccaggaccgctactatagctcatcttggagcgaatgggcatctgtgccctgcagtgttcctggagtaggggtacctggggtgggcgccagaaacctccccgtggccactccagacccaggaatgttcccatgccttcaccactcccaaaacctgctgagggccgtcagcaacatgctccagaaggccagacaaactctagaattttacccttgcacttctgaagagattgatcatgaagatatcacaaaagataaaaccagcacagtggaggcctgtttaccattggaattaaccaagaatgagagttgcctaaattccagagagacctctttcataactaatgggagttgcctggcctccagaaagacctcttttatgatggccctgtgccttagtagtatttatgaagacttgaagatgtaccaggtggagttcaagaccatgaatgcaaagctgctgatggatcctaagaggcagatctttctagatcaaaacatgctggcagttattgatgagctgatgcaggccctgaatttcaacagtgagactgtgccacaaaaatcctcccttgaagaaccggatttttataaaactaaaatcaagctctgcatacttcttcatgctttcagaattcgggcagtgactattgatagagtgatgagctatctgaatgcttcctaa

SEQ ID NO: 4 - protein, 536 aa, synthetic construct
MGHQQLVISWFSLVFLASPLVAIWELKKDVYVVELDWYPDAPGEMVVLTCDTPEEDGITWTLDQSSEVLGSGKTLTIQVKEFGDAGQYTCHKGGEVLSHSLLLLHKKEDGIWSTDILKDQKEPKNKTFLRCEAKNYSGRFTCWWLTTISTDLTFSVKSSRGSSDPQGVTCGAATLSAERVRGDNKEYEYSVECQEDSACPAAEESLPIEVMVDAVHKLKYENYTSSFFIRDIIKPDPPKNLQLKPLKNSRQVEVSWEYPDTWSTPHSYFSLTFCVQVQGKSKREKKDRVFTDKTSATVICRKNASISVRAQDRYYSSSWSEWASVPCSVPGVGVPGVGARNLPVATPDPGMFPCLHHSQNLLRAVSNMLQKARQTLEFYPCTSEEIDHEDITKDKTSTVEACLPLELTKNESCLNSRETSFITNGSCLASRKTSFMMALCLSSIYEDLKMYQVEFKTMNAKLLMDPKRQIFLDQNMLAVIDELMQALNFNSETVPQKSSLEEPDFYKTKIKLCILLHAFRIRAVTIDRVMSYLNAS

SEQ ID NO: 5 - DNA, 20 bp, synthetic construct
  source 1..20: mol_type = other DNA
gctagcctgagatcaccgcg

SEQ ID NO: 6 - DNA, 21 bp, synthetic construct
  source 1..21: mol_type = other DNA
gctagcatccgttgcatccta

SEQ ID NO: 7 - DNA, 8055 bp, synthetic construct
  source 1..8055: mol_type = other DNA
accacaggtgggtgctttggaaacttgtcggtcgccgtgctcctgtgagcttgcgtccctccccggtttcctttgcgctcccgccttccggacctgctctcgcctatcttctttggctgtcggtgcgattcgtcaggcagcggccttgtcgaatctcgaccccaccactcgccggacccgccgacgtcccctctggagcccgccgaaacccgccgcgtctgttgaaatggccagccgcccagccgcatcctctcccgtcgaagcgcgggccccggttgggggacaggaggccggcggccccagcgcagccacccagggggaggccgccggggcccctctcgcccacggccaccacgtgtactgccagcgagtcaatggcgtgatggtgctttccaacaagacgcccgggtccgcgtcctaccgcatcagcgatagcaactttgtccaatgtggttccaactgcaccatgatcatagacggagacgtggtgcgcgggcgcccccaggacccgggggccgcggcatcccccgctcccttcgttgcggtgacaaacatcggagccggcagcgacggcgggaccgccgtcgtggcattcgggggaaccccacgtcgctcggcggggacgtctaccggtacccagacgaccgacgtccccaccgaggcccttgggggcccccctcctcctccccgcttcaccctgggtggcggctgttgttcctgtcgcgacacacggcgccgctctgcggtattcgggggggagggggatcccgtcggccccgcggagttcgtctcggacgaccggtcgtccgattccgactcggatgactcggaggacaccgactcggagacgctgtcacacgcctcctcggacgtgtccggcggggccacgtacgacgacgcccttgactccgattcgtcatcggatgactccctgcagatagatggccccgtgtgtcgcccgtggagcaatgacaccgcgcccctggatgtttgccccgggacccccggcccgggcgccgacgccggtggtccctcagcggtagacccacacgcaccgacgccaggggccggcgctggtcttgcggccgatcccgccgtggcccgggacgacgcggaggggctttcggacccccggccacgtctgggaacgggcacggcctaccccgtccccctggaactcacgcccgagaacgcggaggccgtggcgcgctttctgggagatgccgtgaaccgcgaacccgcgctcatgctggagtacttttgccggtgcgcccgcgaggaaaccaagcgtgtcccccccaggacattctgcagcccccctcgcctcacggaggacgactttgggcttctcaactacgcgctcgtggagatgcagcgcctgtgtctggacgttcctccggtcccgccgaacgcatacatgccctattatctcagggagtatgtgacgcggctggtcaacgggttcaagccgctggtgagccggtccgctcgcctttaccgcatcctgggggttctggtgcacctgcggatccggacccgggaggctagagcggccgcatcgaatataacttcgtataatgtatgctatacgaagttatccatggttgatcccgtcgttttacaacgtcgtgactgggaaaaccctggcgttacccaacttaatcgccttgcagcacatccccctttcgccagctggcgtaatagcgaagaggcccgcaccgatcgcccttcccaacagttgcgcagcctgaatggcgaatggcgctttgcctggtttccggcaccagaagcggtgccggaaagctggctggagtgcgatcttcctgaggccgatactgtcgtcgtcccctcaaactggcagatgcacggttacgatgcgcccatctacaccaacgtgacctatcccattacggtcaatccgccgtttgttcccacggagaatccgacgggttgttactcgctcacatttaatgttgatgaaagctggctacaggaaggccagacgcgaattatttttgatggcgttaactcggcgtttcatctgtggtgcaacgggcgctgggtcggttacggccaggacagtcgtttgccgtctgaatttgacctgagcgcatttttacgcgccggagaaaaccgcctcgcggtgatggtgctgcgctggagtgacggcagttatctggaagatcaggatatgtggcggatgagcggcattttccgtgacgtctcgttgctgcataaaccgactacacaaatcagcgatttccatgttgccactcgctttaatgatgatttcagccgcgctgtactggaggctgaagttcagatgtgcggcgagttgcgtgactacctacgggtaacagtttctttatggcagggtgaaacgcaggtcgccagcggcaccgcgcctttcggcggtgaaattatcgatgagcgtggtggttatgccgatcgcgtcacactacgtctgaacgtcgaaaacccgaaactgtggagcgccgaaatcccgaatctctatcgtgcggtggttgaactgcacaccgccgacggcacgctgattgaagcagaagcctgcgatgtcggtttccgcgaggtgcggattgaaaatggtctgctgctgctgaacggcaagccgttgctgattcgaggcgttaaccgtcacgagcatcatcctctgcatggtcaggtcatggatgagcagacgatggtgcaggatatcctgctgatgaagcagaacaactttaacgccgtgcgctgttcgcattatccgaaccatccgctgtggtacacgctgtgcgaccgctacggcctgtatgtggtggatgaagccaatattgaaacccacggcatggtgccaatgaatcgtctgaccgatgatccgcgctggctaccggcgatgagcgaacgcgtaacgcgaatggtgcagcgcgatcgtaatcacccgagtgtgatcatctggtcgctggggaatgaatcaggccacggcgctaatcacgacgcgctgtatcgctggatcaaatctgtcgatccttcccgcccggtgcagtatgaaggcggcggagccgacaccacggccaccgatattatttgcccgatgtacgcgcgcgtggatgaagaccagcccttcccggctgtgccgaaatggtccatcaaaaaatggctttcgctacctggagagacgcgcccgctgatcctttgcgaatacgcccacgcgatgggtaacagtcttggcggtttcgctaaatactggcaggcgtttcgtcagtatccccgtttacagggcggcttcgtctgggactgggtggatcagtcgctgattaaatatgatgaaaacggcaacccgtggtcggcttacggcggtgattttggcgatacgccgaacgatcgccagttctgtatgaacggtctggtctttgccgaccgcacgccgcatccagcgctgacggaagcaaaacaccagcagcagtttttccagttccgtttatccgggcaaaccatcgaagtgaccagcgaatacctgttccgtcatagcgataacgagctcctgcactggatggtggcgctggatggtaagccgctggcaagcggtgaagtgcctctggatgtcgctccacaaggtaaacagttgattgaactgcctgaactaccgcagccggagagcgccgggcaactctggctcacagtacgcgtagtgcaaccgaacgcgaccgcatggtcagaagccgggcacatcagcgcctggcagcagtggcgtctggcggaaaacctcagtgtgacgctccccgccgcgtcccacgccatcccgcatctgaccaccagcgaaatggatttttgcatcgagctgggtaataagcgttggcaatttaaccgccagtcaggctctctttcacagatgtggattggcgataaaaaccaactgctgacgccgctgcgcgatcagttcacccgtgcaccgctggataacgacattggcgtaagtgaagcgacccgcattgaccctaacgcctgggtcgaacgctggaaggcggcgggccattaccaggccgaagcagcgttgttgcagtgcacggcagatacacttgctgatgcggtgctgattacgaccgctcacgcgtggcagcatcaggggaaaaccttatttatcagccggaaaacctaccggattgatggtagtggtcaaatggcgattaccgttgatgttgaagtggcgagcgatacaccgcatccggcgcggattggcctgaactgccagctggcgcaggtagcagagcgggtaaactggctcggattagggccgcaagaaaactatcccgaccgccttactgccgcctgttttgaccgctgggatctgccattgtcagacatgtataccccgtacgtcttcccgagcgaaaacggtctgcgctgcgggacgcgcgaattgaattatggcccacaccagtggcgcggcgacttccagttcaacatcagccgctacagtcaacagcaactgatggaaaccagccatcgccatctgctgcacgcggaagaaggcacatggctgaatatcgacggtttccatatggggattggtggcgacgactcctggagcccgtcagtatcggcggaattccagctgagcgccggtcgctaccattaccagttggtctggtgtcaaaaaaagggcgaattcggtaagcctatccctaaccctctcctcggtctcgattctacgcgtaccgggtgctacgagatttcgattccaccgccgccttctatgaaaggttgggcttcggaatcgttttccgggacgccggctggatgatcctccagcgcggggatctcatgctggagttcttcgcccaccccaacttgtttattgcagcttataatggttacaaataaagcaatagcatcacaaatttcacaaataaagcatttttttcactgcattctagttgtggtttgtccaaactcatcaatgtatcttatcatgtctgtataccgtcgaggctggttctttccgcctcagaagccatagagcccaccgcatccccagcatgcctgctattgtcttcccaatcctcccccttgctgtcctgccccaccccaccccccagaatagaatgacacctactcagacaatgcgatgcaatttcctcattttattaggaaaggacagtgggagtggcaccttccagggtcaaggaaggcacgggggaggggcaaacaacagatggctggcaactagaaggcacagtcgaggctgatcagcgggtttaaactcaatggtgatggtgatgatgaccggtatgcatattcagatcctcttctgagatgagtttttgttcgaaccgcgggctagcccctccctagttcttaatccacatcctatcaaagtttcctcatttcaaagttttataaaaatgacaacggtttggagggacctcgctttttaggaagcattcagatagctcatcactctatcaatagtcactgcccgaattctgaaagcatgaagaagtatgcagagcttgattttagttttataaaaatccggttcttcaagggaggatttttgtggcacagtctcactgttgaaattcagggcctgcatcagctcatcaataactgccagcatgttttgatctagaaagatctgcctcttaggatccatcagcagctttgcattcatggtcttgaactccacctggtacatcttcaagtcttcataaatactactaaggcacagggccatcataaaagaggtctttctggaggccaggcaactcccattagttatgaaagaggtctctctggaatttaggcaactctcattcttggttaattccaatggtaaacaggcctccactgtgctggttttatcttttgtgatatcttcatgatcaatctcttcagaagtgcaagggtaaaattctagagtttgtctggccttctggagcatgttgctgacggccctcagcaggttttgggagtggtgaaggcatgggaacattcctgggtctggagtggccacggggaggtttctggcgcccaccccaggtacccctactccaggaacactgcagggcacagatgcccattcgctccaagatgagctatagtagcggtcctgggcccgcacgctaatgctggcatttttgcggcagatgaccgtggctgaggtcttgtccgtgaagactctatctttcttttctctcttgctcttgccctggacctgaacgcagaatgtcagggagaagtaggaatgtggagtactccaggtgtcagggtactcccagctgacctccacctgccgagaattctttaatggcttcagctgcaagttcttgggtgggtcaggtttgatgatgtccctgatgaagaagctgctggtgtagttttcatacttgagcttgtgaacggcatccaccatgacctcaatgggcagactctcctcagcagctgggcaggcactgtcctcctggcactccactgagtactcatactccttgttgtcccctctgactctctctgcagagagtgtagcagctccgcacgtcaccccttgggggtcagaagagcctctgctgcttttgacactgaatgtcaaatcagtactgattgtcgtcagccaccagcaggtgaaacgtccagaataattcttggcctcgcatcttagaaaggtcttatttttgggttctttctggtcctttaaaatatcagtggaccaaattccatcttcctttttgtgaagcagcaggagcgaatggcttagaacctcgcctcctttgtgacaggtgtactggccagcatctccaaactctttgacttggatggtcagggttttgccagagcctaagacctcactgctctggtccaaggtccaggtgataccatcttcttcaggggtgtcacaggtgaggaccaccatttctccaggggcatccggataccaatccaattctacgacataaacatctttcttcagttcccatatggccacgaggggagatgccagaaaaaccagggaaaaccaagagatgaccaactgctggtgacccatggtggcgcggccgcttaggcctaacctaggaacccgggaaggatccgagctcggtaccaagcttaactagccagcttgggtctccctatagtgagtcgtattaatttcgataagccagtaagcagtgggttctctagttagccagagagctctgcttatatagacctcccaccgtacacgcctaccgcccatttgcgtcaatggggcggagttgttacgacattttggaaagtcccgttgattttggtgccaaaacaaactcccattgacgtcaatggggtggagacttggaaatccccgtgagtcaaaccgctatccacgcccattgatgtactgccaaaaccgcatcaccatggtaatagcgatgactaatacgtagatgtactgccaagtaggaaagtcccataaggtcatgtactgggcataatgccaggcgggccatttaccgtcattgacgtcaatagggggcgtacttggcatatgatacacttgatgtactgccaagtgggcagtttaccgtaaatactccacccattgacgtcaatggaaagtccctattggcgttactatgggaacatacgtcattattgacgtcaatgggcgggggtcgttgggcggtcagccaggcgggccatttaccgtaagttatgtaacgcggaactccatatatgggctatgaactaatgaccccgtaattgattactattaataactagtcaataatcaatgtcaacgcgtatatctggcccgtacatcgcctgtcgacatttaaatgctagcggtacccttaagcctgcaggactagtactgatccgaagttcctatactttctagagaataggaacttcctcgaggtcatggggttcggcgagcagatacccatccaggagctggcctatggcattgtgcgcagtgcggccacgaccgggagccccttcgtcatgttcaaagacgcggtgaaccgccactacatctacgacacccagggggcggccatcgccggctccaacctc

SEQ ID NO: 8 - DNA, 1449 bp, synthetic construct
  source 1..1449: mol_type = other DNA
agcgagttagacaggcaagcactactcgcctctgcacgcacatgcttgcctgtcaaactctaccaccccggcacgctctctgtctccatggcccgccgccgccgccatcgcggcccccgccgcccccggccgcccgggcccacgggcgccgtcccaaccgcacagtcccaggtaacctccacgcccaactcggaacccgcggtcaggagcgcgcccgcggccgccccgccgccgccccccgccggtgggcccccgccttcttgttcgctgctgctgcgccagtggctccacgttcccgagtccgcgtccgacgacgacgatgacgacgactggccggacagccccccgcccgagccggcgccagaggcccggcccaccgccgccgccccccggccccggcccccaccgcccggcgtgggcccggggggcggggctgacccctcccaccccccctcgcgccccttccgccttccgccgcgcctcgccctccgcctgcgcgtcaccgcggagcacctggcgcgcctgcgcctgcgacgcgcgggcggggagggggcgccggagccccccgcgacccccgcgacccccgcgacccccgcgacccccgcgacccccgcgcgggtgcgcttctcgccccacgtccgggtgcgccacctggtggtctgggcctcggccgcccgcctggcgcgccgcggctcgtgggcccgcgagcgggccgaccgggctcggttccggcgccgggtggcggaggccgaggcggtcatcgggccgtgcctggggcccgaggcccgtgcccgggccctggcccgcggagccggcccggcgaactcggtctaacgttacacccgaggcggcctgggtcttccgcggagctcccgggagctccgcaccaagccgctctccggagagacgatggcaggagccgcgcatatatacgcttggagccagcccgccctcacagggcgggccgcctcgggggcgggactggccaatcggcggccgccagcgcggcggggcccggccaaccagcgtccgccgagtcttcggggcccggcccattgggcgggagttaccgcccaatgggccgggccgcccacttcccggtatggtaattaaaaacttgcaagaggccttgttccgcttcccggtatggtaattagaaactcattaatgggcggccccggccgcccttcccgcttccggcaattcccgcggcccttaatgggcaaccccggtattccccgcctcccgcgccgcgcgtaaccactcccctggggttccgggttatgctaattgcttttttggcggaacacacggcccctcgcgcattggcccgcgggtcgctcaatgaacccgcattggtcccctggggttccgggtatggtaatgagtttcttcgggaaggcgggaagccccggggcaccgacgcaggccaagcccctgttgcgtcgg

SEQ ID NO: 9 - DNA, 707 bp, synthetic construct
  source 1..707: mol_type = other DNA
attatcaccccgttgcgggggtccggagatcatgcgcgggtgtcctcgaggtgcgtgaacacctctggggtgcatgccggcggacggcacgccttttaagtaaacatctgggtcgcccggcccaactggggccgggggttgggtctggctcatctcgagagccacgggggggaaccaccctccgcccagagactcgggtgatggtcgtacccgggactcaacgggttaccggattacggggactgtcggtcacggtcccgccggttcttcgatgtgccacacccaaggatgcgttgggggcgatttcgggcagcagcccgggagagcgcagcaggggacgctccgggtcgtgcacggcggttctggccgcctcccggtcctcacgcccccttttattgatctcatcgcgtacgtcggcgtacgtcctgggcccaacccgcatggtgtccaggaaggtgtccgccatttccagggcccacgacatgctcccccccgacgagcaggaagcggtccacgcaacggtcgccgccggtcgcctcgacgaggacgttcctcctgcgggaaggcacgaacgcgggtgagccccctcctccgcccccgcgtcccccctcctccgcccccgcgtcccccctcctccgcccccgcgtcccccctcctccgcccccgcgtcccccctcctccgcccccgcgtcccccctcctccgccc

SEQ ID NO: 10 - DNA, 19 bp, synthetic construct
  source 1..19: mol_type = other DNA
cgcaaatgggcgtagcgtg

SEQ ID NO: 11 - DNA, 17 bp, synthetic construct
  source 1..17: mol_type = other DNA
tagaggcacagtcgagg

SEQ ID NO: 12 - DNA, 20 bp, synthetic construct
  source 1..20: mol_type = other DNA
acccgcccaagaacttgcag

SEQ ID NO: 13 - DNA, 20 bp, synthetic construct
  source 1..20: mol_type = other DNA
ggatcgaccctgcagggaac